European Patent Specification EP 3 292 872 B9, published August 9, 2023. Title: Compositions for treating or preventing infection-induced inflammatory diseases and for enhancing immune responses comprising tryptophanyl-tRNA synthetase. Applicant: Medicinal Bioconvergence Research Center DAEJEON UNIVERSITY Industry-University Cooperation Foundation. The sequence listing filed with the application follows.

SEQUENCE LISTING (18 sequences)

SEQ ID NO: 1 - protein, 471 aa, Artificial Sequence
  Homo sapiens (Accession No. NP_004175.2)
MPNSEPASLLELFNSIATQGELVRSLKAGNASKDEIDSAVKMLVSLKMSYKAAAGEDYKADCPPGNPAPTSNHGPDATEAEEDFVDPWTVQTSSAKGIDYDKLIVRFGSSKIDKELINRIERATGQRPHHFLRRGIFFSHRDMNQVLDAYENKKPFYLYTGRGPSSEAMHVGHLIPFIFTKWLQDVFNVPLVIQMTDDEKYLWKDLTLDQAYSYAVENAKDIIACGFDINKTFIFSDLDYMGMSSGFYKNVVKIQKHVTFNQVKGIFGFTDSDCIGKISFPAIQAAPSFSNSFPQIFRDRTDIQCLIPCAIDQDPYFRMTRDVAPRIGYPKPALLHSTFFPALQGAQTKMSASDPNSSIFLTDTAKQIKTKVNKHAFSGGRDTIEEHRQFGGNCDVDVSFMYLTFFLEDDDKLEQIRKDYTSGAMLTGELKKALIEVLQPLIAEHQARRKEVTDEIVKEFMTPRKLSFDFQ

SEQ ID NO: 2 - protein, 481 aa, Artificial Sequence
  Rattus norvegicus (Accession No. Q6P7B0.2)
MADMPSGESCTSPLELFNSIAAQGELVRSLKAGNAPKDEIESAVKMLLSLKMNYKTAMGEEYKAGCPPGNSTAGSNGDPDATKASEDFVDPWTVRTSSAKGIDYDKLIVQFGSSKIDKELINRIERATGQRPHRFLRRGIFFSHRDMNQILDAYENKKPFYLYTGRGPSSEAMHLGHLVPFIFTKWLQDVFDVPLVIQMSDDEKYLWKDLTLEQAYSYTVENAKDIIACGFDVNKTFIFSDLEYMGQSPGFYKNVVKIQKHVTFNQVKGIFGFTDSDCIGKISFPAVQAAPSFSNSFPKIFRDRTDIQCLIPCAIDQDPYFRMTRDVAPRIGHPKPALLHSTFFPALQGAQTKMSASDPNSSIFLTDTAKQIKSKVNKHAFSGGRDTVEEHRQFGGNCEVDVSFMYLTFFLEDDDSLEQIRKDYTSGAMLTGELKKTLIDVLQPLIAEHQARRKAVTEETVKEFMAPRQLSFHFQCFCFDT

SEQ ID NO: 3 - protein, 481 aa, Artificial Sequence
  Mus musculus (Accession No. P32921.2)
MADMPSGESCTSPLELFNSIATQGELVRSLKAGNAPKDEIDSAVKMLLSLKMSYKAAMGEEYKAGCPPGNPTAGRNCDSDATKASEDFVDPWTVRTSSAKGIDYDKLIVQFGSSKIDKELINRIERATGQRPHRFLRRGIFFSHRDMNQILDAYENKKPFYLYTGRGPSSEAMHLGHLVPFIFTKWLQDVFNVPLVIQMSDDEKYLWKDLTLEQAYSYTVENAKDIIACGFDINKTFIFSDLEYMGQSPGFYRNVVKIQKHVTFNQVKGIFGFTDSDCIGKISFPAVQAAPSFSNSFPKIFRDRTDIQCLIPCAIDQDPYFRMTRDVAPRIGHPKPALLHSTFFPALQGAQTKMSASDPNSSIFLTDTAKQIKSKVNKHAFSGGRDTVEEHRQFGGNCEVDVSFMYLTFFLEDDDRLEQIRKDYTSGAMLTGELKKTLIDVLQPLIAEHQARRKAVTEETVKEFMTPRQLSFHFQCFCFDT

SEQ ID NO: 4 - protein, 476 aa, Artificial Sequence
  Bos taurus (Accession No. P17248.3)
MADMSNGEQGCGSPLELFHSIAAQGELVRDLKARNAAKDEIDSAVKMLLSLKTSYKAATGEDYKVDCPPGDPAPESGEGLDATEADEDFVDPWTVQTSSAKGIDYDKLIVRFGSSKIDKELVNRIERATGQRPHRFLRRGIFFSHRDMHQILDAYENKKPFYLYTGRGPSSEAMHVGHLIPFIFTKWLQDVFNVPLVIQMTDDEKYLWKDLTLDQAYGYAVENAKDIIACGFDINKTFIFSDLDYMGMSPGFYKNVVKIQKHVTFNQVKGIFGFTDSDCIGKISFPAIQAAPSFSNSFPQIFRDRTDVQCLIPCAIDQDPYFRMTRDVAPRIGYPKPALLHSTFFPALQGAQTKMSASDPNSSIFLTDTAKQIKTKVNKHAFSGGRDTVEEHRQFGGNCDVDVSFMYLTFFLEDDDKLEQIRRDYTSGAMLTGELKKELIEVLQPLIAEHQARRKEVTDEIVKEFMTPRKLSYDFQ

SEQ ID NO: 5 - protein, 476 aa, Artificial Sequence
  Sus scrofa (Accession No. JAA53775.1)
MADVPNGEQGCSSPLELFNSIAAQGELVRSLKARHAAKDEIDSAVKMLLSLKMSYKAAMGEDYKADCPPGNRAPGIDSGLDATEAGDDFVDPWTVQTSSAKGIDYDKLIVRFGSSKIDKELIDRIERATGQRPHRFLRRGIFFSHRDMNQVLDAYENKKPFYLYTGRGPSSEAMHVGHLIPFIFTKWLQDVFNVPLVIQMTDDEKYLWKELTLEQAHGYAVENAKDIIACGFDVNKTFIFSDLDYMGMSPGFYKNVVKIQKHVTFNQVKGIFGFTDSDCIGKISFPAIQAAPSFSSSFPQIFRDRTDIQCLIPCAIDQDPYFRMTRDVAPRIGYPKPALLHSTFFPALQGAQTKMSASDPNSSIFLTDTAKQIKTKVNKHAFSGGRDTIEEHRQFGGNCDVDVSFMYLTFFLEDDDRLEQIRKDYSSGAMLTGELKKVLIEVLQPLIAEHQARRKEVTDEVVKEFMTPRKLSYDFE

SEQ ID NO: 6 - protein, 476 aa, Artificial Sequence
  Ovis aries (Accession No. XP_004018038.1)
MADMPNGEQGYGSPLELFHSIAAQGELVRGLKARNAAKDEIDSAVKMLLSLKTSYKAATGEDYKGDHPPEDPAPESGEGLDATGADEDFVDPWTVQTSSAKGIDYDKLIVRFGSSKIDKELVNRIERATGQRPHRFLRRGIFFSHRDMHQILDAYENKKPFYLYTGRGPSSEAMHVGHLIPFIFTKWLQDVFNVPLVIQMTDDEKYLWKDLTLDQAYGYAVENAKDIIACGFDINKTFIFSDLDYMGMSPGFYKNVVKIQKHVTFNQVKGIFGFTDSDCIGKISFPAIQAAPSFSNSFPQIFRDRTDVQCLIPCAIDQDPYFRMTRDVAPRIGYPKPALLHSTFFPALQGAQTKMSASDPNSSIFLTDTAKQIKTKVNKHAFSGGRDTIEEHRQLGGNCDVDVSFMYLTFFLEDDDRLEQIRKDYTSGAMLTGELKKELIEVLQPLIAEHQARRKEVTDEIVKEFMTPRKLSYDFQ

SEQ ID NO: 7 - protein, 476 aa, Artificial Sequence
  Canis lupus (Accession No. XP_537554.1)
MADMPNGEQGFASPLELFNSIAAQGELVRSLKAGKASKDEIDSAVKLLLSLKMSYKATVGEEYKADCPPARPAPENSRGLNAAEAEEDFVDPWTVQTSSAKGIDYDKLIVRFGSSKIDKELVNRIERATGQKPHRFLRRGIFFSHRDMNQILDAYENKKPFYLYTGRGPSSEAMHVGHLIPFIFTKWLQDVFNVPLVIQMTDDEKYLWKDLTLDQAYGYAVENAKDIIACGFDIKKTFIFSDLDYMGMSPGFYKNVVKIQKHVTFNQVKGIFGFTDSDSIGKISFPAIQAAPSFSNSFPQIFRDRTDIQCLIPCAIDQDPYFRMTRDVAPRIGYPKPALLHSTFFPALQGAQTKMSASDPNSSIFLTDTAKQIKTKVNKHAFSGGRDTIEEHRQFGGNCDVDVSFMYLTFFLEDDDKLEQIRKDYTSGDMLTGELKKTLIEVLQPLIAEHQARRKEVTDEIVKEFMTPRKLSYDFQ

SEQ ID NO: 8 - protein, 476 aa, Artificial Sequence
  Felis catus (Accession No. XP_003988038.1)
MADVPNGEQGCASPLELFNRIAAQGELVRSLKAGKAPQDEIDSAVQMLLSLKMSYKAAMGEDYKADCPPGNPAPGNNSGLGATEAEEDFVDPWTVQTSSAKGIDYDKLIVRFGSSKIDKELVNRIERAIGQKPHRFLRRGIFFSHRDMNQILDAYENKKPFYLYTGRGPSSEAMHVGHLIPFIFTKWLQDVFNVPLVIQMTDDEKYLWKDLTLDQAYGYAVENAKDIIACGFDINKTFIFSDLDYMGASPGFYKNVVKIQKHVTFNQVKGIFGFTDSDSIGKISFPAIQAAPSFSNSFPQIFGDKTDVQCLIPCAIDQDPYFRMTRDVAPRIGYPKPALLHSTFFPALQGAQTKMSASDPNSSIFLTDTAKQIKTKVNKHAFSGGRDTVEEHREFGGNCDVDVSFMYLTFFLEDDDRLEQIRKDYTSGAMLTGELKKILIEVLQPLIAEHQARRKEVTDEIVKEFMTPRKLSYDFQ

SEQ ID NO: 9 - DNA, 20 bp, Artificial Sequence
  hTNF-alpha Forward
ggagaagggtgaccgactca

SEQ ID NO: 10 - DNA, 17 bp, Artificial Sequence
  hTNF-alpha Reverse
ctgcccagactcggcaa

SEQ ID NO: 11 - DNA, 26 bp, Artificial Sequence
  hTrpRS Forward
aagaattcatgcccaacagtgagccc

SEQ ID NO: 12 - DNA, 32 bp, Artificial Sequence
  hTrpRS Reverse
aactcgagctaccctggaggacagtcagcctt

SEQ ID NO: 13 - DNA, 21 bp, Artificial Sequence
  GAPDH forward
cgctctctgctcctcctgttc

SEQ ID NO: 14 - DNA, 22 bp, Artificial Sequence
  GAPDH reverse
ttgactccgaccttcaccttcc

SEQ ID NO: 15 - DNA, 20 bp, Artificial Sequence
  hMIP-1 alpha Forward
accatggctctctgcaacca

SEQ ID NO: 16 - DNA, 20 bp, Artificial Sequence
  hMIP-1 alpha Reverse
ttaagaagagtcccacagtg

SEQ ID NO: 17 - DNA, 21 bp, Artificial Sequence
  hMIP-1 beta Forward
agcctcacctctgagaaaacc

SEQ ID NO: 18 - DNA, 22 bp, Artificial Sequence
  hMIP-1 beta Reverse
gcaacagcagagaaacagtgac